European Patent Application EP 4 148 131 A1, published March 15, 2023. Title: RNA for inhibiting SARS-CoV-2 replication. Applicant: Charité - Universitätsmedizin Berlin Technische Universität Berlin Freie Universität Berlin. The sequence listing filed with the application follows.

SEQUENCE LISTING (12 sequences)

SEQ ID NO: 1 - DNA, 21 bp, Artificial Sequence
  siRNA
  misc_feature (20)..(21): single-stranded overhanging nucleotides
uuauacugcgugagugcactt

SEQ ID NO: 2 - DNA, 21 bp, Artificial Sequence
  siRNA
  misc_feature (20)..(21)
  misc_feature (20)..(21): single-stranded overhanging nucleotides
gauagacgaguuacucgugtt

SEQ ID NO: 3 - DNA, 21 bp, Artificial Sequence
  siRNA
  misc_feature (20)..(21): single-stranded overhanging nucleotides
uuaccuuucggucacaccctt

SEQ ID NO: 4 - DNA, 21 bp, Artificial Sequence
  siRNA
  misc_feature (20)..(21): single-stranded overhanging nucleotides
uuacucguguccugucaactt

SEQ ID NO: 5 - DNA, 21 bp, Artificial Sequence
  siRNA
  misc_feature (20)..(21): single-stranded overhanging nucleotides
aguuacucguguccugucatt

SEQ ID NO: 6 - DNA, 21 bp, Artificial Sequence
  siRNA
  misc_feature (20)..(21): single-stranded overhanging nucleotides
uucguuuagagaacagauctt

SEQ ID NO: 7 - DNA, 21 bp, Artificial Sequence
  siRNA
  misc_feature (20)..(21): single-stranded overhanging nucleotides
uaccuuucggucacacccgtt

SEQ ID NO: 8 - DNA, 21 bp, Artificial Sequence
  siRNA
  misc_feature (20)..(21): single-stranded overhanging nucleotides
gagaucgaaaguugguuggtt

SEQ ID NO: 9 - DNA, 21 bp, Artificial Sequence
  siRNA
  misc_feature (20)..(21): single-stranded overhanging nucleotides
acgugacacguucggagaatt

SEQ ID NO: 10 - DNA, 57 bp, Artificial Sequence
  shRNA
gttgacaggacacgagtaagccctgacccagcttactcgtgtcctgtcaactttttt

SEQ ID NO: 11 - DNA, 57 bp, Artificial Sequence
  shRNA
gatctgttctctaaacgaagccctgacccagcttcgtttagagaacagatctttttt

SEQ ID NO: 12 - DNA, 57 bp, Artificial Sequence
  shRNA
ggggtgtgaccgaaaggtagccctgacccagctacctttcggtcacacccctttttt